European Patent Specification EP 4 504 761 B1, published February 4, 2026. Title: NOVEL RECOMBINANT SPIDER SILK-REINFORCED COLLAGEN PROTEINS PRODUCED IN PLANTS AND THE USE THEREOF. Applicant: SwiftPharma BV. The sequence listing filed with the application follows.

SEQUENCE LISTING (20 sequences)

SEQ ID NO: 1 - protein, 1057 aa, synthetic construct
QLSYGYDEKSTGGISVPGPMGPSGPRGLPGPPGAPGPQGFQGPPGEPGEPGASGPMGPRGPPGPPGKNGDDGEAGKPGRPGERGPPGPQGARGLPGTAGLPGMKGHRGFSGLDGAKGDAGPAGPKGEPGSPGENGAPGQMGPRGLPGERGRPGAPGPAGARGNDGATGAAGPPGPTGPAGPPGFPGAVGAKGEAGPQGPRGSEGPQGVRGEPGPPGPAGAAGPAGNPGADGQPGAKGANGAPGIAGAPGFPGARGPSGPQGPGGPPGPKGNSGEPGAPGSKGDTGAKGEPGPVGVQGPPGPAGEEGKRGARGEPGPTGLPGPPGERGGPGSRGFPGADGVAGPKGPAGERGSPGPAGPKGSPGEAGRPGEAGLPGAKGLTGSPGSPGPDGKTGPPGPAGQDGRPGPPGPPGARGQAGVMGFPGPKGAAGEPGKAGERGVPGPPGAVGPAGKDGEAGAQGPPGPAGPAGERGEQGPAGSPGFQGLPGPAGPPGEAGKPGEQGVPGDLGAPGPSGARGERGFPGERGVQGPPGPAGPRGANGAPGNDGAKGDAGAPGAPGSQGAPGLQGMPGERGAAGLPGPKGDRGDAGPKGADGSPGKDGVRGLTGPIGPPGPAGAPGDKGESGPSGPAGPTGARGAPGDRGEPGPPGPAGFAGPPGADGQPGAKGEPGDAGAKGDAGPPGPAGPAGPPGPIGNVGAPGAKGARGSAGPPGATGFPGAAGRVGPPGPSGNAGPPGPPGPAGKEGGKGPRGETGPAGRPGEVGPPGPPGPAGEKGSPGADGPAGAPGTPGPQGIAGQRGVVGLPGQRGERGFPGLPGPSGEPGKQGPSGASGERGPPGPMGPPGLAGPPGESGREGAPGAEGSPGRDGSPGAKGDRGETGPAGPPGAPGAPGAPGPVGPAGKSGDRGETGPAGPAGPVGPVGARGPAGPQGPRGDKGETGEQGDRGIKGHRGFSGLQGPPGPPGSPGEQGPSGASGPAGPRGPPGSAGAPGKDGLNGLPGPIGPPGPRGRTGDAGPVGPPGPPGPPGPPGPPSAGFDFSFLPQPPQEKAHDGGRYYRA

SEQ ID NO: 2 - protein, 1040 aa, synthetic construct
QYDGKGVGLGPGPMGLMGPRGPPGAAGAPGPQGFQGPAGEPGEPGQTGPAGARGPAGPPGKAGEDGHPGKPGRPGERGVVGPQGARGFPGTPGLPGFKGIRGHNGLDGLKGQPGAPGVKGEPGAPGENGTPGQTGARGLPGERGRVGAPGPAGARGSDGSVGPVGPAGPIGSAGPPGFPGAPGPKGEIGAVGNAGPAGPAGPRGEVGLPGLSGPVGPPGNPGANGLTGAKGAAGLPGVAGAPGLPGPRGIPGPVGAAGATGARGLVGEPGPAGSKGESGNKGEPGSAGPQGPPGPSGEEGKRGPNGEAGSAGPPGPPGLRGSPGSRGLPGADGRAGVMGPPGSRGASGPAGVRGPNGDAGRPGEPGLMGPRGLPGSPGNIGPAGKEGPVGLPGIDGRPGPIGPAGARGEPGNIGFPGPKGPTGDPGKNGDKGHAGLAGARGAPGPDGNNGAQGPPGPQGVQGGKGEQGPPGPPGFQGLPGPSGPAGEVGKPGERGLHGEFGLPGPAGPRGERGPPGESGAAGPTGPIGSRGPSGPPGPDGNKGEPGVVGAVGTAGPSGPSGLPGERGAAGIPGGKGEKGEPGLRGEIGNPGRDGARGAPGAVGAPGPAGATGDRGEAGAAGPAGPAGPRGSPGERGEVGPAGPNGFAGPAGAAGQPGAKGERGAKGPKGENGVVGPTGPVGAAGPAGPNGPPGPAGSRGDGGPPGMTGFPGAAGRTGPPGPSGISGPPGPPGPAGKEGLRGPRGDQGPVGRTGEVGAVGPPGFAGEKGPSGEAGTAGPPGTPGPQGLLGAPGILGLPGSRGERGLPGVAGAVGEPGPLGIAGPPGARGPPGAVGSPGVNGAPGEAGRDGNPGNDGPPGRDGQPGHKGERGYPGNIGPVGAAGAPGPHGPVGPAGKHGNRGETGPSGPVGPAGAVGPRGPSGPQGIRGDKGEPGEKGPRGLPGLKGHNGLQGLPGIAGHHGDQGAPGSVGPAGPRGPAGPSGPAGKDGRTGHPGTVGPAGIRGPQGHQGPAGPPGPPGPPGPPGVSGGGYDFGYDGDFYRA

SEQ ID NO: 3 - DNA, 3174 bp, synthetic construct
  source 1..3174: mol_type = other DNA
cagttgtcttatggttatgatgaaaaatcaactggaggaattagtgttccaggtccaatgggaccatctggaccaagaggtcttcctggacctccaggtgctcctggtccacagggttttcagggaccaccaggagaaccaggagagccaggagcttcaggtcctatgggtccaagaggtccacctggccctccaggaaagaatggtgatgatggagaagcaggaaagcctggtcgtccaggcgaaagaggtcctcctggaccacaaggggctagaggactgcctggtactgctggacttccaggaatgaaaggtcatagaggtttttctggacttgacggtgctaagggagatgcaggaccagctggacctaagggtgagccaggatctccaggcgagaacggagcccctggtcagatgggaccaagaggattgccaggtgaaagaggaaggcctggagctcctggtccagctggagctaggggtaatgatggagctactggagctgcaggacctcctggtccaactggtcctgctggaccaccaggttttcctggagctgtgggagctaaaggtgaggctggtccacaaggtcctagaggatcagaaggaccccaaggagttagaggagaaccaggtccacctggaccagccggtgcagctggtcctgctggtaatcctggtgctgacggacaacctggcgctaaaggtgcaaacggagctcctggaatcgcaggtgctccaggttttccaggtgcaagaggtcctagtggtccacagggtccaggaggtccaccaggaccaaagggtaatagtggtgagcctggagctccaggaagcaaaggagatactggtgctaagggcgaaccaggaccagttggagtgcaaggacctccaggaccagcaggagaagaaggtaagagaggagctaggggagaaccaggacctactggtttgccaggaccaccaggtgaacgtggaggacctggatcaaggggttttccaggagctgatggggttgctggtcctaagggaccagcaggagaaagaggatctccaggtcctgctggaccaaaaggaagtcctggagaagctggcagacctggagaagcaggtcttccaggtgctaagggtcttactggatctccaggatctcctggtcctgatggaaaaactggaccaccaggtcctgctggacaagacggtagacctggacctcctggtccacctggagctagaggtcaagctggtgttatgggatttcctggaccaaagggtgctgctggtgaaccagggaaagctggtgaaagaggagtgcctggtccacctggagctgttggccctgctggaaaggatggtgaagctggtgctcaaggaccaccaggacctgctggtcctgctggagaaagaggtgagcagggaccagctggaagtcctggttttcaaggattgccaggaccagctggtcctccaggggaagcaggtaagccaggcgaacaaggagtcccaggagatttgggagctcctggaccatctggagcaagaggtgaaagaggatttccaggagaaagaggagttcagggtccgccaggacctgctggaccaagaggagcaaacggagcaccaggaaatgatggagctaagggggatgctggtgctccaggtgcacctggatctcaaggagctccaggactccaaggaatgcctggtgaaagaggtgctgctggtcttccaggacctaagggagatagaggagatgcaggaccaaagggagctgatggaagccctggtaaggatggtgttagaggacttactggaccaataggtcctcctggtccagctggagcacctggggataagggtgagagtggtccttctggtcctgcaggcccaacaggagcaagaggtgctcctggtgatagaggtgaacctggacctccaggtcctgctggatttgctggtccacctggtgctgatggacaacctggagcaaagggagagcctggagatgcaggagcaaaaggagatgctggtccacctggaccagctggtcctgctggtcctcctggaccaatcggtaatgttggagctcctggtgctaaaggtgctaggggttcagctggacctcctggagctactggttttcctggtgctgctggcagggttggaccacctggtccaagtggaaatgccggaccacctggcccaccaggaccagctggaaaagaaggtggaaaaggaccaagaggagaaactggtccagcaggtcgtccaggtgaagtgggccctccaggcccaccaggacctgctggagaaaagggaagtccaggtgcagatggaccagctggcgctcctggtactccaggacctcagggtatcgctggacaaagaggtgttgttggtttgccaggtcagagaggagagagaggttttccaggattgccaggtccttctggtgagcctggtaaacagggtccttctggagcttctggtgaaagaggacctcctggtcctatgggtccaccaggattggcaggaccaccaggtgaatctggaagagaaggtgcaccaggagcagaaggatctccaggtagggatggaagccctggggctaaaggagataggggagaaactggaccagcaggaccaccaggtgctcctggtgccccaggtgctcctggaccagttggtcctgctggtaagtctggtgacagaggtgaaactgggccagctggaccagctggacctgttggtcctgttggtgctagaggtccagctggacctcaaggtcctagaggagataaaggagaaactggtgaacaaggtgataggggtattaagggtcataggggattttctggtttgcaaggaccacctggaccaccaggttcaccaggagagcaaggtccaagtggagcatctggaccagctggtccaaggggacctcctggatctgctggagctccaggtaaagatggacttaatggtcttccaggtccaattggacctcctggaccaagaggaagaactggagatgcaggaccagttggaccaccaggtccaccaggacctcctggtcctccaggacctccaagtgcaggttttgatttttcatttcttcctcaaccaccacaagagaaggctcacgatggaggaaggtattatagagcttaa

SEQ ID NO: 4 - DNA, 3123 bp, synthetic construct
  source 1..3123: mol_type = other DNA
caatacgatggaaaaggagttggtctcggaccaggtccaatgggtttgatgggaccaagaggtcctccaggagctgctggtgctcctggtcctcaaggatttcaaggaccagctggagagccaggtgagcctggacagactggtccagctggtgcaagaggacctgcaggacctcccggtaaagctggtgaagatggacatccaggaaaaccaggaagaccaggagagaggggtgtcgttggaccacaaggtgcaagaggttttccaggaacaccaggtcttcctggttttaaaggtattagagggcacaatggtttggatggtttgaagggtcaaccaggtgctccaggagttaaaggagaacctggtgctccaggtgaaaatggtactccgggacaaactggagcaagaggattgcctggagaaaggggtcgtgttggtgcaccaggtcctgcaggagcaagaggttcagatggatctgtgggtccagttggtcctgctggaccaattggttctgctggtcctcctggatttccaggagctcctggaccaaagggagaaattggagcagttggaaatgcaggacctgctggtcctgctggacctagaggtgaagttggattgcctggtttgtcgggcccagtaggtcctccaggaaatccaggagctaatggattgactggtgctaaaggagctgctggattgcctggtgtggcaggtgctcctggtcttccaggtcctagaggcattcctggtccagtaggagctgcaggagctactggtgcaagaggtcttgttggagaaccaggacccgcaggttcaaaaggagaatctggaaataaaggtgaaccaggatctgctggacctcagggtccacctggtcctagtggtgaagaaggaaagagaggacctaatggtgaggccggaagcgctggtcctcctggaccaccaggtcttagaggaagtcctggtagtagaggattgccaggagcagatggaagagctggtgttatgggaccaccaggttctagaggagctagcggaccagctggagtgaggggtccaaatggagatgctggaaggcctggagaaccaggattgatgggtcctaggggtttaccaggaagtccaggaaatattggaccagcaggtaaagaaggacctgtgggtttgccaggaattgatggaaggccaggaccaattggaccagctggtgctagaggagagcctggtaatattggttttccaggtccaaagggtccaactggagaccctggaaagaacggtgataaaggacatgcaggacttgctggagcaagaggagctcctggccctgatggtaataatggtgctcaaggtcctccaggaccacaaggtgttcaaggaggaaaaggtgagcaaggaccacctggaccaccaggttttcaaggacttcctggcccatctggtccagctggtgaagttggaaaaccaggagagagaggtcttcatggagaatttggacttccaggaccagctggccctagaggagaaagaggacctccaggtgaatctggtgctgcaggtccaactggaccaattggttccagaggaccatccggacctcctggaccagatggaaataaaggtgaaccaggagttgtgggtgctgttggtacagcaggtccatcaggtccatctggtcttccaggagagaggggcgctgctggtattcctggtggaaagggagagaagggcgaaccaggactcagaggtgaaattggaaatcccggaagagatggagcaagaggagctcctggagctgttggtgctccaggaccagctggtgcaacaggtgataggggtgaagctggggctgctggacctgctggaccagctggtcctaggggttctcctggagaaagaggtgaggtaggtcctgctggacctaatggttttgctgggccagccggtgctgctggacaaccaggagccaagggagagagaggagctaaaggaccaaaaggagagaatggagtcgttggtcctactggaccagttggagctgctggaccagctggaccaaatggaccaccaggaccagctggatctagaggagatggtggaccaccaggtatgacaggtttcccaggtgcagctggaaggactggacctccagggccatcaggtatttctggacctccaggaccaccaggtccagctggaaaagagggtctcagaggaccaagaggagatcaaggaccagtgggaagaacaggtgaagtgggtgctgtgggtccacctggttttgctggggagaaaggtccttccggagaagctggaactgcaggtccaccaggaactccaggtccacagggtttgcttggagctcctggaattcttggtttacctggttcaagaggagaaagaggtcttcctggtgttgctggagccgttggagagccaggaccattgggaattgctggacctccaggtgctaggggaccacctggcgctgtgggatctccaggcgtgaatggtgcaccaggagaggcaggaagggatggtaatccgggtaacgatggacctccaggtagagatgggcaaccaggacacaagggggaaaggggttatccaggaaatattggacctgttggagctgcaggtgctccaggtcctcatggaccagttggacctgcaggaaaacatggaaatagaggagagactggtccttcaggtcctgtgggaccagcaggtgctgttggtcctagaggtccatcaggaccacaaggtattagaggagataagggagagccaggagaaaagggaccaagaggtttacctggtttgaaaggacataatggattgcaggggcttccaggtattgctggccatcacggtgatcagggagctccaggttctgtaggtccagcaggtccaaggggaccagctggtccttctggacctgctggtaaggatggtaggactggtcatccaggaactgtgggaccagcaggaattaggggtcctcaagggcatcaaggtcctgctggtccacctggacctccaggtcctccaggacctcctggtgtttctggtggtgggtatgattttggttacgatggagatttttatagggcatga

SEQ ID NO: 5 - protein, 748 aa, synthetic construct
QGAGAAAAAAGGAGQGGYGGLGGQGAGQGGYGGLGGQGAGQGAGAAAAAAAGGAGQGGYGGLGSQGAGRGGQGAGAAAAAAGGAGQGGYGGLGSQGAGRGGLGGQGAGAAAAAAAGGAGQGGYGGLGNQGAGRGGQGAAAAAAGGAGQGGYGGLGSQGAGRGGLGGQGAGAAAAAAGGAGQGGYGGLGGQGAGQGGYGGLGSQGAGRGGLGGQGAGAAAAAAAGGAGQGGLGGQGAGQGAGASAAAAGGAGQGGYGGLGSQGAGRGGEGAGAAAAAAGGAGQGGYGGLGGQGAGQGGYGGLGSQGAGRGGLGGQGAGAAAAGGAGQGGLGGQGAGQGAGAAAAAAGGAGQGGYGGLGSQGAGRGGLGGQGAGAVAAAAAGGAGQGGYGGLGSQGAGRGGQGAGAAAAAAGGAGQRGYGGLGNQGAGRGGLGGQGAGAAAAAAAGGAGQGGYGGLGNQGAGRGGQGAAAAAGGAGQGGYGGLGSQGAGRGGQGAGAAAAAAVGAGQEGIRGQGAGQGGYGGLGSQGSGRGGLGGQGAGAAAAAAGGAGQGGLGGQGAGQGAGAAAAAAGGVRQGGYGGLGSQGAGRGGQGAGAAAAAAGGAGQGGYGGLGGQGVGRGGLGGQGAGAAAAGGAGQGGYGGVGSGASAASAAASRLSSPQASSRVSSAVSNLVASGPTNSAALSSTISNVVSQIGASNPGLSGCDVLIQALLEVVSALIQILGSSSIGQVNYGSAGQATQIVGQSVYQALG

SEQ ID NO: 6 - DNA, 2247 bp, synthetic construct
  source 1..2247: mol_type = other DNA
caaggagctggagctgcagctgcagctgctggaggagctggacaaggtggatatggtggtttgggaggtcaaggtgctggacaaggaggttacggaggtcttggaggacagggagctggacaaggtgctggtgctgcagctgctgctgctgctggaggagctggtcaaggaggttacggtggtttaggttcacaaggagctggtagaggaggacagggtgcaggtgctgctgctgcagcagcaggaggtgctggacagggcggttatggtggtttgggttcccaaggagctggaaggggaggattaggtggacagggagctggtgctgctgctgctgctgctgcaggaggtgctggtcagggtggctatggtggtttggggaatcaaggagctggaaggggtggtcaaggagctgcagcagctgctgctggaggtgctggacaaggcggttacggaggtttgggatctcagggtgcaggaagaggaggtcttggcggacagggagctggagctgctgccgctgctgctggaggtgcaggacaaggcggttatggtggtcttggtggtcaaggagcaggacaaggtgggtacgggggacttggaagtcagggtgctggtaggggaggacttggaggacaaggtgctggggcagctgctgcagctgctgctggaggtgctggacaaggaggtcttggtggacagggagcaggacaaggtgctggagcatctgcagctgcagcaggtggagcagggcagggaggatacggaggacttggttctcaaggtgctggtagaggaggtgaaggagcaggtgctgctgcagctgcagctggaggcgctggacaaggaggctatggaggacttggtggacagggggctggacagggtggttatggaggtcttggatcccagggagctgggaggggaggactcggaggacaaggagctggagctgcagctgctggtggtgctggacaaggtggacttggtggacaaggagctggccaaggtgctggagctgcagctgctgctgctggtggtgcaggtcaaggaggatatggaggacttggaagtcaaggagctggaagaggaggtcttggtggtcaaggtgccggagcagttgctgccgctgctgctggaggtgctggtcagggtggatatggaggtcttggttctcagggtgcaggaagaggaggtcaaggagcaggtgctgcagctgcagctgcaggtggagctggtcaaagaggatacggaggacttggaaaccagggtgctggtagaggaggccttggaggtcagggagctggggctgctgctgctgctgcagctggtggtgctggacaaggtggatatggtggactcggaaatcagggtgctggaagaggtggacaaggtgctgcagctgcagctggcggagcaggacaaggtggatatggtggtttgggttcacagggagcaggaagaggaggacagggagctggtgctgctgctgcagcagctgttggagcaggacaagaaggaattagaggacaaggagctggtcagggaggatatggaggtttgggatctcaaggttcaggtaggggtggacttggtggacaaggagcaggagcagctgctgctgctgctggtggagctggacaaggaggattgggaggacaaggagctggtcaaggagctggagctgctgccgcagctgctggaggagtgagacaaggtgggtatggtggtttgggttcacaaggagcaggtagaggtggacaaggagcaggtgcagcagcagcagctgctggtggtgctggtcaaggaggttacggtggacttggaggtcaaggagttggtaggggaggtcttggtggtcaaggggctggtgctgctgccgctggtggagctggacaaggtggttatggtggtgttggttctggagcttctgctgctagtgctgctgcatcaagactttcttctcctcaagcttcttctagagttagcagcgctgttagtaaccttgtagcttcaggtccaactaattctgctgctctttctagtactatttctaatgttgtgagccaaatcggagcttcaaatccaggattgtctggttgtgatgttttaattcaagctttgttggaggtggtttctgctcttattcagattttgggttcttcttctatcggtcaagttaactatggatctgctggtcaggctacacaaattgttggtcagtctgtttaccaggctcttgggtga

SEQ ID NO: 7 - protein, 636 aa, synthetic construct
ARAGSGQQGPGQQGPGQQGPGQQGPYGPGASAAAAAAGGYGPGSGQQGPSQQGPGQQGPGGQGPYGPGASAAAAAAGGYGPGSGQQGPGGQGPYGPGSSAAAAAAGGNGPGSGQQGAGQQGPGQQGPGASAAAAAAGGYGPGSGQQGPGQQGPGGQGPYGPGASAAAAAAGGYGPGSGQGPGQQGPGGQGPYGPGASAAAAAAGGYGPGSGQQGPGQQGPGQQGPGGQGPYGPGASAAAAAAGGYGPGYGQQGPGQQGPGGQGPYGPGASAASAASGGYGPGSGQQGPGQQGPGGQGPYGPGASAAAAAAGGYGPGSGQQGPGQQGPGQQGPGQQGPGGQGPYGPGASAAAAAAGGYGPGSGQQGPGQQGPGQQGPGQQGPGQQGPGQQGPGQQGPGQQGPGQQGPGGQGAYGPGASAAAGAAGGYGPGSGQQGPGQQGPGQQGPGQQGPGQQGPGQQGPGQQGPGQQGPYGPGASAAAAAAGGYGPGSGQQGPGQQGPGQQGPGGQGPYGPGAASAAVSVGGYGPQSSSVPVASAVASRLSSPAASSRVSSAVSSLVSSGPTKHAALSNTISSVVSQVSASNPGLSGCDVLVQALLEVVSALVSILGSSSIGQINYGASAQYTQMVGQSVAQALA

SEQ ID NO: 8 - DNA, 1911 bp, synthetic construct
  source 1..1911: mol_type = other DNA
gcaagagcaggatctggtcagcaaggacctggtcaacaaggtccaggacagcagggaccaggacaacaaggtccttatggacctggtgcttcagcagctgctgctgctgctggtggttatggaccaggatctggacaacagggcccttctcagcaaggacctggacagcagggtcctggtggtcaaggaccttacggtcctggagcttctgctgctgctgctgctgcaggtggatatggtcctggtagtggtcaacaaggtccaggaggacaaggaccatacggccctggtagctcagctgctgcagcagctgctggtggtaatggcccaggaagtggacaacaaggtgctggacaacagggtccaggacaacaaggacctggtgcatcagccgctgctgctgctgctggaggttatggaccaggttctggacaacaaggtccaggacaacaaggaccaggaggtcaaggaccttatggaccaggagctagtgctgcagcagctgctgctggaggttatggtcctggaagtggtcaaggacctggacaacaaggacctgggggtcaaggtccttatggacctggagcttccgctgctgctgcagcagccggaggttatggtccaggaagtggtcagcaaggaccaggacagcagggaccaggacagcaaggtcctggaggtcagggaccatatggtccaggagcttctgctgctgctgcagctgctggtggatatggaccaggttatggacaacaaggacctggacaacaaggacctggagggcaaggtccatatggaccaggagcttctgctgctagtgctgcttcaggagggtatggaccaggttctggacaacaaggaccaggacaacaaggtccaggtggtcaaggaccttatggaccgggtgcttctgcagctgccgcagctgctggaggatatggtcctggttcaggtcaacaaggacccggtcaacaaggaccaggtcagcaaggtccaggacaacagggtcctggaggtcagggtccttatgggccaggagcatctgctgcagctgctgctgctggtggttatggaccaggctctggacaacaaggacctggtcaacaaggacctggacagcagggtcctggacagcaaggtccaggacaacaaggaccaggacagcaaggtccaggtcagcaaggacctggacaacaaggaccaggtcaacaaggacctggtggtcagggtgcttatggtccaggtgctagtgctgctgccggagcagctggaggctatggacctggatctggtcagcagggacctggtcaacaaggacctggtcaacagggaccaggtcaacaaggaccagggcaacagggacctggacaacaaggacctggacaacaaggtccaggtcagcagggaccttatggacctggtgcttcagctgctgctgcagctgctggaggatatggcccaggttctggacaacagggacctggacaacaaggtccaggtcaacaaggtccaggtggccaaggaccatacggaccaggagctgcatctgcagctgtttctgttggaggatatggacctcaatcatcatctgttcctgtggcatcagctgttgcttcaagattgtcttcaccagctgcttcatctagagttagcagtgcagtttcttccttggtttcttctggacctactaaacatgctgctctctctaatactattagtagtgttgtttctcaggtttctgcttctaatccaggtttatcaggatgcgatgttcttgttcaagcacttttggaagttgtttccgctttggtttcaattttaggatcatcttctattggtcaaattaattatggcgcttctgcccaatatactcagatggtcggacaatcagttgctcaagctcttgcttaa

SEQ ID NO: 9 - protein, 284 aa, synthetic construct
MDISNLPPHIRQQILGLISKPQQNNDESSSSNNKNNLINNEKVSNVLIDLTSNLKIENFKIFNKESLNQLEKKGYLIIDNFLNDLNKINLIYDESYNQFKENKLIEAGMNKGTDKWKDKSIRGDYIQWIHRDSNSRIQDKDLSSTIRNINYLLDKLDLIKNEFDNVIPNFNSIKTQTQLAVYLNGGRYIKHRDSFYSSESLTISRRITMIYYVNKDWKKGDGGELRLYTNNPNNTNQKELKQTEEFIDIEPIADRLLIFLSPFLEHEVLQCNFEPRIAITTWIY

SEQ ID NO: 10 - protein, 490 aa, synthetic construct
APDEEDHVLVLHKGNFDEALAAHKYLLVEFYAPWCGHCKALAPEYAKAAGKLKAEGSEIRLAKVDATEESDLAQQYGVRGYPTIKFFKNGDTASPKEYTAGREADDIVNWLKKRTGPAASTLSDGAAAEALVESSEVAVIGFFKDMESDSAKQFFLAAEVIDDIPFGITSNSDVFSKYQLDKDGVVLFKKFDEGRNNFEGEVTKEKLLDFIKHNQLPLVIEFTEQTAPKIFGGEIKTHILLFLPKSVSDYEGKLSNFKKAAESFKGKILFIFIDSDHTDNQRILEFFGLKKEECPAVRLITLEEEMTKYKPESDELTAEKITEFCHRFLEGKIKPHLMSQELPDDWDKQPVKVLVGKNFEEVAFDEKKNVFVEFYAPWCGHCKQLAPIWDKLGETYKDHENIVIAKMDSTANEVEAVKVHSFPTLKFFPASADRTVIDYNGERTLDGFKKFLESGGQDGAGDDDDLEDLEEAEEPDLEEDDDQKAVKDEL

SEQ ID NO: 11 - DNA, 855 bp, synthetic construct
  source 1..855: mol_type = other DNA
atggatatttctaatttgccaccacatatcaggcagcaaattcttggcttgatttctaagccacaacaaaataacgatgagagttcttcatcaaacaataaaaataaccttattaacaacgagaaggtgtcaaatgttttgattgatcttacttccaatcttaagattgagaacttcaaaatctttaacaaggagtctctcaatcagcttgaaaagaagggataccttattattgataatttcttgaatgatttgaataaaattaatttaatttatgatgaatcctataatcaatttaaagaaaataaacttatagaagctggaatgaacaagggaactgataagtggaaagataagtcaatcagaggagattacatacagtggattcatcgggattctaatagtagaattcaggataaggatctttcatctacgattagaaatattaattatcttctcgataaacttgacttgattaaaaatgagtttgataatgtcattccaaattttaattcaatcaaaacacaaactcaattagcagtgtacttgaatggcggtaggtacattaagcatagagattctttctattcttctgaaagtcttactatttctaggaggattactatgatatactatgtgaataaggattggaagaagggagatggaggtgagttgagattgtatacaaacaatccaaataatacaaatcaaaaagagttgaagcagactgaagaattcattgatattgaacctattgctgatcgtttacttatttttctttcccccttccttgaacatgaggtgcttcaatgcaatttcgagccaaggatagctattactacttggatatactaa

SEQ ID NO: 12 - DNA, 1473 bp, synthetic construct
  source 1..1473: mol_type = other DNA
gctcctgatgaagaggaccatgtacttgttttgcataagggtaattttgatgaagctcttgcagcacataaatatctattggtggagttctatgcaccttggtgtggacactgcaaggctttggctccagagtacgctaaggctgcaggaaaacttaaggctgagggttctgagattagactcgctaaggttgatgctactgaggaatcagatttggctcagcaatatggagttaggggatacccaactattaaatttttcaaaaatggggatactgcatcaccaaaagaatacactgccgggagagaagctgatgatattgttaattggttgaagaagaggactggccctgctgcttctactttgtctgatggagcagctgcagaggcacttgttgaatcttcagaagttgctgttattggatttttcaaagatatggagtccgattctgctaagcaattctttctggcagcagaagtcattgatgatattccatttggaatcacttcaaattctgatgttttttctaagtatcagcttgataaggatggggttgttctttttaaaaaattcgacgagggaaggaataacttcgagggagaggtgacaaaagagaagcttcttgatttcattaagcataatcagctccctcttgttattgaatttaccgaacagactgcacctaagatcttcggtggagaaattaaaactcatattttgctttttttgccaaaatctgtttcagattatgaaggaaaactttctaattttaagaaagctgctgaatcatttaagggtaagattttgtttatttttattgactcagatcatactgataatcaaaggatcttggaattttttgggttaaagaaggaggaatgtcctgctgttagacttattactttggaggaagaaatgacaaagtacaagcctgaaagtgatgaattgacagcagaaaagattactgaattctgtcatcgtttcctggaaggtaagattaagccacatttgatgtcccaagaacttcctgatgattgggataagcaacctgttaaggttctcgttggtaagaattttgaagaggtggcttttgatgagaaaaagaatgtctttgttgagttctatgcaccttggtgtggacactgtaaacaattggctccaatttgggacaagctcggtgaaacctataaggatcacgaaaacattgttattgctaagatggattctacagctaatgaagtggaggctgttaaggtgcattcttttccaacacttaaatttttcccagcttcagctgataggactgtaatagattataacggagagcgtactctagatggtttcaaaaagtttctggagtcaggtggtcaagatggagctggagatgatgatgatcttgaagatctcgaggaagctgaggaaccagatcttgaggaggatgatgatcaaaaagctgttaaggatgagttgtga

SEQ ID NO: 13 - protein, 722 aa, synthetic construct
SDRPRGRDPVNPEKLLVITVATAETEGYLRFLRSAEFFNYTVRTLGLGEEWRGGDVARTVGGGQKVRWLKKEMEKYADREDMIIMFVDSYDVILAGSPTELLKKFVQSGSRLLFSAESFCWPEWGLAEQYPEVGTGKRFLNSGGFIGFATTIHQIVRQWKYKDDDDDQLFYTRLYLDPGLREKLSLNLDHKSRIFQNLNGALDEVVLKFDRNRVRIRNVAYDTLPIVVHGNGPTKLQLNYTYPEHERELGNYVPNGWTPEGGCGFCNQDRRTLPGGQPPPRVFLAVFVEQPTPFLPRFLQRLLLLDYPPDRVTLFLHNNEVFHEPHIADSWPQLQDHFSAVKLVGPEEALSPGEARDMAMDLCRQDPECEFYFSLDADAVLTNLQTLRILIEENRKVIAPMLSRHGKLWSNFWGALSPDEYYARSEDYVELVQRKRVGVWNVPYISQAYVIRGDTLRMELPQRDVFSGSDTDPDMAFCKSFRDKGIFLHLSNQHEFGRLLATSRYDTEHLHPDLWQIFDNPVDWKEQYIHENYSRALEGEGIVEQPCPDVYWFPLLSEQMCDELVAEMEHYGQWSGGRHEDSRLAGGYENVPTVDIHMKQVGYEDQWLQLLRTYVGPMTESLFPGYHTKARAVMNFVVRYRPDEQPSLRPHHDSSTFTLNVALNHKGLDYEGGGCRFLRYDCVISSPRKGWALLHPGRLTHYHEGLPTTWGTRYIMVSFVDP

SEQ ID NO: 14 - DNA, 2145 bp, synthetic construct
  source 1..2145: mol_type = other DNA
tctgataggccacgtggaagagatcctgtgaacccagagaagcttttggttattactgttgctactgcagagactgaaggataccttagatttcttcgttcagcagagttctttaattatactgttagaactttgggattgggtgaagaatggagaggaggagatgttgctaggactgttggtggtggacaaaaagttaggtggttgaagaaggaaatggaaaagtatgctgatagggaggatatgattattatgtttgtggattcctatgacgttattcttgctggatctcctaccgagcttcttaaaaagtttgttcaatcaggatcaagacttctctttagtgcagagagtttctgttggccagaatggggtctcgctgaacaatacccagaagttggaactggaaagagattcttgaattctggaggatttattggatttgctacaactattcatcaaattgttagacagtggaagtataaggatgatgatgatgatcagcttttttatactaggctttatttagatcctggtctcagagaaaaactttctttgaatcttgatcataagagcagaatcttccaaaatcttaacggagctttggatgaggttgttcttaaatttgatagaaacagagttaggattagaaatgttgcttatgatactttgcctattgttgttcatggaaatggaccaactaagcttcaacttaactatcttggtaactacgttcctaatggatggactccagaaggtggttgtggattttgcaaccaggatagaaggacacttcctgggggacaaccccctccaagggtgttcttggctgtttttgttgaacaaccaactccatttttgcctcgttttttgcaaagactgctacttcttgattatccacctgatagagttactttgttcttgcataataatgaagtttttcatgaaccacatattgcagattcttggccacaactccaagatcactttagcgctgttaaacttgttggtccagaagaagctttgtctcctggtgaagcaagagacatggccatggatctctgcagacaagacccagaatgtgaattttattttagtttggatgctgatgctgttttgactaatttgcagacattgagaattcttatcgaagaaaacaggaaagttattgctcccatgctttcaaggcatggaaagctctggtctaatttctggggtgcactttctccagacgaatactatgcaagatctgaagattatgttgagttggttcagagaaagagagttggagtttggaacgttccctatatttcacaggcttacgttattagaggagataccttgcgtatggaattgccacagagggatgttttctctggctctgatacagatccagatatggctttctgcaaatcttttagagacaaaggtatttttttgcatttgtcaaaccaacatgaattcggtagacttcttgctacctctaggtatgatactgaacaccttcatccagatctctggcaaatttttgacaatcctgttgactggaaggagcaatatattcacgagaactactctagagctcttgaaggagagggtattgttgagcaaccttgccctgatgtgtactggtttcctttgctctctgagcaaatgtgtgatgaacttgttgctgaaatggaacattacggccaatggtcaggtggtaggcatgaggattcaagacttgctggtggttacgaaaacgttccaacagtggatatccatatgaagcaagttggttatgaagatcagtggcttcaattgcttaggacttatgttggacctatgactgaatcactttttccaggatatcacacaaaggctagagctgtgatgaattttgttgttagatatagaccagatgaacagccatcattgagaccacatcatgattcttctacttttactttaaatgtggctcttaaccataagggactggattacgaaggaggaggttgcagatttcttagatatgattgtgttatttcctctccaagaaaagggtgggcattgttacatccaggtagacttacacattaccatgaaggacttcctactacttggggaactcgttatattatggtttctttcgttgatccttaa

SEQ ID NO: 15 - protein, 2943 aa, synthetic construct
MATTLISKLTLSSAFLGQQFSSRGNSMRSAPAGLFLRGPRQGAGAAAAAAGGAGQGGYGGLGGQGAGQGGYGGLGGQGAGQGAGAAAAAAAGGAGQGGYGGLGSQGAGRGGQGAGAAAAAAGGAGQGGYGGLGSQGAGRGGLGGQGAGAAAAAAAGGAGQGGYGGLGNQGAGRGGQGAAAAAAGGAGQGGYGGLGSQGAGRGGLGGQGAGAAAAAAGGAGQGGYGGLGGQGAGQGGYGGLGSQGAGRGGLGGQGAGAAAAAAAGGAGQGGLGGQGAGQGAGASAAAAGGAGQGGYGGLGSQGAGRGGEGAGAAAAAAGGAGQGGYGGLGGQGAGQGGYGGLGSQGAGRGGLGGQGAGAAAAGGAGQGGLGGQGAGQGAGAAAAAAGGAGQGGYGGLGSQGAGRGGLGGQGAGAVAAAAAGGAGQGGYGGLGSQGAGRGGQGAGAAAAAAGGAGQRGYGGLGNQGAGRGGLGGQGAGAAAAAAAGGAGQGGYGGLGNQGAGRGGQGAAAAAGGAGQGGYGGLGSQGAGRGGQGAGAAAAAAVGAGQEGIRGQGAGQGGYGGLGSQGSGRGGLGGQGAGAAAAAAGGAGQGGLGGQGAGQGAGAAAAAAGGVRQGGYGGLGSQGAGRGGQGAGAAAAAAGGAGQGGYGGLGGQGVGRGGLGGQGAGAAAAGGAGQGGYGGVGSGASAASAAASRLSSPQASSRVSSAVSNLVASGPTNSAALSSTISNVVSQIGASNPGLSGCDVLIQALLEVVSALIQILGSSSIGQVNYGSAGQATQIVGQSVYQALGGSGEGRGSLLTCEDVEENPGPQLSYGYDEKSTGGISVPGPMGPSGPRGLPGPPGAPGPQGFQGPPGEPGEPGASGPMGPRGPPGPPGKNGDDGEAGKPGRPGERGPPGPQGARGLPGTAGLPGMKGHRGFSGLDGAKGDAGPAGPKGEPGSPGENGAPGQMGPRGLPGERGRTYPEHEREPGAPGPAGARGNDGATGAAGPPGPTGPAGPPGFPGAVGAKGEAGPQGPRGSEGPQGVRGEPGPPGPAGAAGPAGNPGADGQPGAKGANGAPGIAGAPGFPGARGPSGPQGPGGPPGPKGNSGEPGAPGSKGDTGAKGEPGPVGVQGPPGPAGEEGKRGARGEPGPTGLPGPPGERGGPGSRGFPGADGVAGPKGPAGERGSPGPAGPKGSPGEAGRPGEAGLPGAKGLTGSPGSPGPDGKTGPPGPAGQDGRPGPPGPPGARGQAGVMGFPGPKGAAGEPGKAGERGVPGPPGAVGPAGKDGEAGAQGPPGPAGPAGERGEQGPAGSPGFQGLPGPAGPPGEAGKPGEQGVPGDLGAPGPSGARGERGFPGERGVQGPPGPAGPRGANGAPGNDGAKGDAGAPGAPGSQGAPGLQGMPGERGAAGLPGPKGDRGDAGPKGADGSPGKDGVRGLTGPIGPPGPAGAPGDKGESGPSGPAGPTGARGAPGDRGEPGPPGPAGFAGPPGADGQPGAKGEPGDAGAKGDAGPPGPAGPAGPPGPIGNVGAPGAKGARGSAGPPGATGFPGAAGRVGPPGPSGNAGPPGPPGPAGKEGGKGPRGETGPAGRPGEVGPPGPPGPAGEKGSPGADGPAGAPGTPGPQGIAGQRGVVGLPGQRGERGFPGLPGPSGEPGKQGPSGASGERGPPGPMGPPGLAGPPGESGREGAPGAEGSPGRDGSPGAKGDRGETGPAGPPGAPGAPGAPGPVGPAGKSGDRGETGPAGPAGPVGPVGARGPAGPQGPRGDKGETGEQGDRGIKGHRGFSGLQGPPGPPGSPGEQGPSGASGPAGPRGPPGSAGAPGKDGLNGLPGPIGPPGPRGRTGDAGPVGPPGPPGPPGPPGPPSAGFDFSFLPQPPQEKAHDGGRYYRAGSGEGRGSLLTCEDVEENPGPQYDGKGVGLGPGPMGLMGPRGPPGAAGAPGPQGFQGPAGEPGEPGQTGPAGARGPAGPPGKAGEDGHPGKPGRPGERGVVGPQGARGFPGTPGLPGFKGIRGHNGLDGLKGQPGAPGVKGEPGAPGENGTPGQTGARGLPGERGRVGAPGPAGARGSDGSVGPVGPAGPIGSAGPPGFPGAPGPKGEIGAVGNAGPAGPAGPRGEVGLPGLSGPVGPPGNPGANGLTGAKGAAGLPGVAGAPGLPGPRGIPGPVGAAGATGARGLVGEPGPAGTYPEHERESKGESGNKGEPGSAGPQGPPGPSGEEGKRGPNGEAGSAGPPGPPGLRGSPGSRGLPGADGRAGVMGPPGSRGASGPAGVRGPNGDAGRPGEPGLMGPRGLPGSPGNIGPAGKEGPVGLPGIDGRPGPIGPAGARGEPGNIGFPGPKGPTGDPGKNGDKGHAGLAGARGAPGPDGNNGAQGPPGPQGVQGGKGEQGPPGPPGFQGLPGPSGPAGEVGKPGERGLHGEFGLPGPAGPRGERGPPGESGAAGPTGPIGSRGPSGPPGPDGNKGEPGVVGAVGTAGPSGPSGLPGERGAAGIPGGKGEKGEPGLRGEIGNPGRDGARGAPGAVGAPGPAGATGDRGEAGAAGPAGPAGPRGSPGERGEVGPAGPNGFAGPAGAAGQPGAKGERGAKGPKGENGVVGPTGPVGAAGPAGPNGPPGPAGSRGDGGPPGMTGFPGAAGRTGPPGPSGISGPPGPPGPAGKEGLRGPRGDQGPVGRTGEVGAVGPPGFAGEKGPSGEAGTAGPPGTPGPQGLLGAPGILGLPGSRGERGLPGVAGAVGEPGPLGIAGPPGARGPPGAVGSPGVNGAPGEAGRDGNPGNDGPPGRDGQPGHKGERGYPGNIGPVGAAGAPGPHGPVGPAGKHGNRGETGPSGPVGPAGAVGPRGPSGPQGIRGDKGEPGEKGPRGLPGLKGHNGLQGLPGIAGHHGDQGAPGSVGPAGPRGPAGPSGPAGKDGRTGHPGTVGPAGIRGPQGHQGPAGPPGPPGPPGPPGVSGGGYDFGYDGDFYRA

SEQ ID NO: 16 - DNA, 8784 bp, synthetic construct
  source 1..8784: mol_type = other DNA
atggctaccactcttatatctaagttgactctttcatcagctttccttggacaacagttttcatctagaggtaattcaatgagatcagcaccagctggactttttcttaggggaccaagacaaggagcaggtgctgctgcagcagcagctggaggtgctggacaaggtggttatggaggacttggaggacaaggagcaggacagggtggatatggtggattgggaggacaaggtgctggacaaggagctggagctgctgctgctgcagcagctggaggtgctggtcagggtggatatggaggattgggaagccaaggagctggtaggggtggtcaaggagctggtgctgctgctgcagcagctggtggagcaggtcagggcggttatggaggcttgggttctcaaggagctggaaggggtggcttgggtggccaaggtgccggtgctgctgctgctgctgctgctggtggtgctggtcaaggcggatatggaggacttggaaaccaaggtgctggccgtggtggacagggagctgctgctgctgctgcaggaggagctggtcagggtgggtatggtggtttgggttcacagggagctggaaggggtggacttggaggacagggtgcaggagcagctgctgctgcagctggtggtgcaggtcaaggtggatacggtggtcttggtggacaaggagctggtcagggtggctacggtggacttggaagtcaaggagctggaagaggtggtcttggaggtcaaggagccggtgctgctgctgcagctgcagctggtggagctggacaaggcggtctgggtggccaaggtgctggacagggagcaggtgcatctgcagctgcagctggtggagctggtcaaggtggctatggtggattgggttctcagggagctggtagaggtggagaaggagctggagctgctgcagctgctgctggaggagcaggtcagggtggttacggaggtttaggaggtcaaggagccggacaaggaggatatggaggtcttggttctcaaggggcagggagaggaggtttaggtggacagggagctggtgctgcagctgctggaggagctggtcagggaggacttggaggacaaggtgcaggtcaaggtgctggtgcagctgctgctgccgctggaggtgctggacagggagggtatggaggccttggtagccagggtgcaggcaggggaggtttgggaggacagggtgctggtgctgtggcagcagctgccgcaggaggtgctggacaaggaggatatggaggacttggatctcaaggtgctggtagaggtggtcaaggagctggagctgctgctgctgcagctggaggagccggtcaaagaggatacggtggactaggtaatcaaggagctggaaggggaggattgggtggtcagggagctggagcagcagctgcagcagctgctggaggagcaggtcaggggggttatggaggattggggaatcaaggtgcaggaagaggtggacaaggggctgctgcagctgctggtggagctggccaaggaggttacggtggacttggttctcagggagcaggaagaggagggcagggagctggagctgcagctgctgctgctgttggtgctggtcaggaaggtattagaggacagggagctggtcaaggaggttacggaggtttagggtcccagggttctggaagaggaggactgggaggacaaggagcaggtgctgctgctgctgcagctggtggtgctggacaaggaggtcttggaggacaaggagctggacagggagctggtgcagctgctgctgctgctggaggagttagacagggaggatatggaggtttgggatcacaaggtgcaggaagaggtggacagggagctggagctgcagctgctgcggctggtggggctggacaaggtggatatggagggcttggaggccaaggagttggaaggggtgggcttggtggacaaggtgcaggtgctgctgctgctggaggtgctggtcaaggcggttacggaggtgttggttctggagcttcagctgcaagtgctgcagctagtaggctttctagtccacaagcatcatctagagtttcttctgctgtttctaatttggtggcatctggtccaacaaactcggcagcactttcttctactatttctaatgttgtttctcagataggtgcatctaacccaggtctttcaggatgtgatgttttgatacaggctttgcttgaagtggttagtgctcttatacaaattctcggatcctcatcaattggtcaagtgaactacggttctgctggacaagctacacagattgttggtcaatcagtttatcaagcacttgggggttctggtgaaggaaggggtagtcttcttacttgtgaagatgtggaagaaaatcctggaccacagctttcttatggatacgatgaaaagtctactggaggtatatctgttcctggtcctatgggacctagtggtcctagaggtttgccaggacctcctggtgctccaggaccacaaggatttcagggaccaccaggggaaccaggtgaacctggagcttctggaccaatgggtcctagaggtccacctggacctcctggtaaaaatggagatgatggtgaggctggaaagccaggaaggccaggagaaagaggtccaccaggaccacagggtgctcgtggtcttccaggaacagccggtttacctggcatgaagggacatagaggattttcaggtttggatggagctaaaggagatgctggaccagctggacctaaaggagagccaggatctcctggagagaatggtgcacctggccagatgggtccaaggggtcttccaggtgagagaggtagacctggagccccaggtccagcaggcgctagagggaatgacggagccacaggtgcagctggtccacctggacctactggtcctgctgggcctcctggctttcctggagctgtaggtgctaagggtgaggctggacctcaaggtcctcgaggatcagaaggtccacaaggagttaggggagagcctggcccaccaggtccagctggagctgcaggtcctgctggtaatccaggagctgatggacaacctggagctaaaggtgctaacggagctcctggaattgctggagcaccaggttttcctggtgctagaggaccatcaggaccacaaggaccaggtggtcctccaggacctaaaggtaatagtggagaaccaggtgctcctggttctaaaggagatactggtgctaagggagaaccaggccctgttggagtccaaggtccacctggaccagctggagaagaaggaaagaggggagctagaggcgaaccaggacctactggattgccaggtcctccaggtgaaagaggaggtccaggttctaggggtttcccaggagcagatggagtagctggacctaagggacccgctggtgaaagaggttcacctggacctgcaggtcctaagggttcaccaggtgaagcaggtagacctggtgaagcaggtttgcctggagctaagggtttgacaggaagtccagggtcacctggaccagatggaaagacaggacctcctggtccagctggtcaagatggaagacctggtcctccaggaccaccaggtgcaagaggacaagctggagttatgggttttcctggtccaaagggagctgctggagagccaggtaaagctggtgaaagaggtgttccaggtcctcctggtgctgttggaccagctggtaaagatggagaagctggagctcaaggtccacctggtcctgcaggaccagctggagaaagaggcgaacaaggtcctgctggttcgccaggatttcagggtttaccaggtcccgctggtcctccaggtgaagctggaaaacctggagaacaaggtgtgcctggagatttgggagctccaggaccttctggtgcaagaggtgagcgtggtttccctggagaaaggggtgttcaaggtccacctggacctgctggtcctagaggagctaacggagctccaggaaatgatggtgcaaagggtgatgctggtgcacctggtgctcctggatctcaaggtgctccaggtcttcagggtatgccaggagagaggggagctgctggattacctgggcctaaaggtgatagaggagatgctggtccaaagggtgctgatggtagtccaggtaaagatggtgttagaggacttacaggccctattggtccacctgggccagctggtgcaccaggtgataagggagaaagtggaccaagtggaccagcaggaccaaccggtgctagaggagcaccaggtgatagaggagaaccaggtccaccaggaccagctggttttgctggtcctccaggagctgatggacaaccaggagctaaaggtgagcctggagatgctggagctaaaggagatgctggtccaccgggaccagcaggtccagcaggcccaccaggtccaattggaaacgttggtgcacctggcgctaagggtgccagaggaagcgcaggtccaccaggagcaactggctttccaggtgctgcaggtagagttggaccaccaggaccttctggaaacgctggacctcctgggcctccaggacctgctggaaaggaaggagggaagggtcctaggggagagactggaccagctggtagaccaggtgaggttggaccaccaggtcctccaggcccagctggtgaaaagggtagtcccggtgctgatggaccagcaggagctccaggaacaccaggacctcaaggtattgctggtcaaagaggtgttgttggtttgcctggtcagagaggagaaagaggatttccaggattgccaggaccttctggtgagcctggtaaacagggtccatcaggtgcttctggggaaagaggaccacctggtcctatgggaccaccaggtttggctggtcctcctggtgaatcaggtagggaaggagctcccggagctgaaggatcaccaggaagagatggatctcctggagctaaaggagatagaggagaaacaggtccagctggaccaccaggagcacctggtgctcctggtgctcctggacctgttggtccagctggtaaatcaggagatagaggtgaaactggacctgctggaccagctggtccagttggacctgttggtgctagagggccagcaggaccacagggtcctagaggagataagggagagactggtgaacaaggagatagaggaatcaaaggtcatagaggatttagtggacttcaaggaccacctggccctcctggttctcctggagaacaaggcccatctggtgcttctggacctgctggcccaaggggaccacctggatctgctggtgcccctggtaaagatggacttaatggattgccaggtccaattggtcctcctggtccaagaggaaggacaggagatgctggacctgttggtcctcctgggccaccaggaccacctggacctcctggacctccaagtgctggttttgatttctcttttttaccacagccaccacaggaaaaagctcatgatggtggaagatactatagagctggttcaggtgagggtagaggatccttacttacatgtgaagatgttgaggaaaatcctggaccacagtacgatggaaaaggtgttggacttggtccaggtccaatgggattgatgggaccaagaggacctccaggagctgcaggagctccaggaccacagggatttcaaggtcctgcaggagagcctggagagccaggtcaaactggacctgcaggagctagaggtccagctggacctccaggtaaagctggagaagatggtcatccaggaaagccagggaggccaggtgaaaggggtgttgttggtccacagggggctagaggcttccctggtacacctggtcttccaggatttaaaggtattagaggtcataatggtttagatggattgaagggtcaaccaggagctccaggtgttaagggggaaccaggagcaccaggtgaaaatggaactcctggtcagactggagctagaggacttccaggagaaagaggtagagtgggtgcacctggtccagcaggggctcgtggtagtgatggttccgttggacccgtcggacctgcaggtccaattggatcagcaggaccacctggattcccaggagctccaggtccaaaaggcgagattggtgctgttggaaatgctgggcctgctggacctgctggtcctagaggagaggttggacttccaggtttgtccggaccagtgggaccacctggaaatccaggagctaatggtcttactggagctaaaggagctgcagggttgcctggtgttgctggagctccaggacttcctggacctagaggaattcctggtccagttggagctgctggtgctactggtgctagaggacttgttggagaaccaggtccagcaggatctaagggagagtcaggtaataaaggtgagccaggaagtgctggtccacaaggtccaccaggaccttctggtgaggagggtaagaggggtccaaatggtgaagctggatcagctggacctccaggaccacctggacttaggggtagccctggttcaagaggactgcctggggctgatggaagagctggagttatgggacctcccggtagtaggggagcatccggaccagctggagtaaggggacctaatggtgatgctggaagaccaggagaacctggattaatgggtcctaggggtctcccaggatctccaggtaacattggtcctgctggtaaagaaggaccagttggtcttccaggcattgatggtagaccaggaccaattgggccagctggtgctcgtggcgaacctggtaatataggattcccaggtcctaagggaccaaccggtgatccaggtaaaaatggtgataaaggtcatgctggattggccggagctaggggagctccaggtccagatggaaataatggtgctcagggaccaccaggaccacagggtgttcaaggtggaaaaggagaacagggtcctcctggtcctccaggtttccaaggacttcctggaccttctggtccagcaggtgaggttggtaaaccaggagagagaggattgcacggagaatttggtttgccaggaccggctggtcctaggggtgaaagaggaccacctggtgaatctggagctgctggaccaactggtcctattggttcaaggggaccttctggacctccaggtccagatggaaataaaggagagccaggagtggttggagctgttggaacagctggaccaagtggaccttcaggactcccaggagagaggggcgctgctggtattcctggtggaaaaggtgagaagggtgagcctggacttagaggagaaataggaaatccaggcagggatggtgcacggggagctcctggagctgttggtgccccaggaccagccggagcaacaggagataggggagaggctggtgctgctggtccagctggacctgcaggacctaggggttcaccaggagaaagaggtgaggttggtccagctggtcctaatggatttgctggtcctgctggtgctgctggtcaacctggagctaagggtgagaggggtgcaaaaggacctaaaggtgaaaatggtgttgttggtcctactggaccagttggagctgctggacctgctggaccaaatggtccacctggtccagctggttctagaggagatggtgggccacctggaatgactggattcccaggtgctgctggaaggactggaccaccaggccctagtggaatttctggaccacctggtcctcctggaccagcaggtaaggaaggtttgaggggaccaagaggggatcagggacctgtaggtagaactggtgaggttggtgctgttggcccaccaggtttcgctggcgaaaagggaccttcaggtgaagctggtacagctggtcctcctggtactcctggtccacaaggtttgcttggtgctcctggtattcttggtcttccaggttcaagaggtgagagaggtcttcctggagtggctggagctgttggagaaccaggtccattgggtatagctggacctccaggcgctagaggcccacctggtgcagtcggatcaccaggtgttaacggagctccaggtgaggcaggtagagatggaaatcctggaaatgatgggcctcctggtagggatggacagccaggtcataaaggtgaaagaggataccctggaaatatcggtcctgttggtgctgctggtgcaccaggaccacatggtcctgttggtcctgctggaaagcatggtaatcgaggagaaactggaccatctggaccagttggtccagcaggtgctgttggaccacgaggaccttcaggaccacagggaattaggggtgataagggcgagcctggtgaaaagggacctaggggtcttccaggtttgaaaggtcataacggactgcaaggacttccaggaattgctggtcaccacggtgatcaaggagccccaggttctgttggtccagctggaccaagaggaccagcaggtccatcaggtccagctggaaaagatggtagaactggacatccaggcacagttggtccagctggtattaggggacctcaaggtcatcaaggaccagctggacctccaggaccacctggtccaccaggaccaccaggtgtttctggaggaggctacgattttggttatgatggtgatttttatagggcttaa

SEQ ID NO: 17 - protein, 1578 aa, synthetic construct
MATTLISKLTLSSAFLGQQFSSRGNSMRSAPAGLFLRGPRMDISNLPPHIRQQILGLISKPQQNNDESSSSNNKNNLINNEKVSNVLIDLTSNLKIENFKIFNKESLNQLEKKGYLIIDNFLNDLNKINLIYDESYNQFKENKLIEAGMNKGTDKWKDKSIRGDYIQWIHRDSNSRIQDKDLSSTIRNINYLLDKLDLIKNEFDNVIPNFNSIKTQTQLAVYLNGGRYIKHRDSFYSSESLTISRRITMIYYVNKDWKKGDGGELRLYTNNPNNTNQKELKQTEEFIDIEPIADRLLIFLSPFLEHEVLQCNFEPRIAITTWIYGSGEGRGSLLTCEDVEENPGPAPDEEDHVLVLHKGNFDEALAAHKYLLVEFYAPWCGHCKALAPEYAKAAGKLKAEGSEIRLAKVDATEESDLAQQYGVRGYPTIKFFKNGDTASPKEYTAGREADDIVNWLKKRTGPAASTLSDGAAAEALVESSEVAVIGFFKDMESDSAKQFFLAAEVIDDIPFGITSNSDVFSKYQLDKDGVVLFKKFDEGRNNFEGEVTKEKLLDFIKHNQLPLVIEFTEQTAPKIFGGEIKTHILLFLPKSVSDYEGKLSNFKKAAESFKGKILFIFIDSDHTDNQRILEFFGLKKEECPAVRLITLEEEMTKYKPESDELTAEKITEFCHRFLEGKIKPHLMSQELPDDWDKQPVKVLVGKNFEEVAFDEKKNVFVEFYAPWCGHCKQLAPIWDKLGETYKDHENIVIAKMDSTANEVEAVKVHSFPTLKFFPASADRTVIDYNGERTLDGFKKFLESGGQDGAGDDDDLEDLEEAEEPDLEEDDDQKAVKDELGSGEGRGSLLTCEDVEENPGPSDRPRGRDPVNPEKLLVITVATAETEGYLRFLRSAEFFNYTVRTTYPEHERELGLGEEWRGGDVARTVGGGQKVRWLKKEMEKYADREDMIIMFVDSYDVILAGSPTELLKKFVQSGSRLLFSAESFCWPEWGLAEQYPEVGTGKRFLNSGGFIGFATTIHQIVRQWKYKDDDDDQLFYTRLYLDPGLREKLSLNLDHKSRIFQNLNGALDEVVLKFDRNRVRIRNVAYDTLPIVVHGNGPTKLQLNYLGNYVPNGWTPEGGCGFCNQDRRTLPGGQPPPRVFLAVFVEQPTPFLPRFLQRLLLLDYPPDRVTLFLHNNEVFHEPHIADSWPQLQDHFSAVKLVGPEEALSPGEARDMAMDLCRQDPECEFYFSLDADAVLTNLQTLRILIEENRKVIAPMLSRHGKLWSNFWGALSPDEYYARSEDYVELVQRKRVGVWNVPYISQAYVIRGDTLRMELPQRDVFSGSDTDPDMAFCKSFRDKGIFLHLSNQHEFGRLLATSRYDTEHLHPDLWQIFDNPVDWKEQYIHENYSRALEGEGIVEQPCPDVYWFPLLSEQMCDELVAEMEHYGQWSGGRHEDSRLAGGYENVPTVDIHMKQVGYEDQWLQLLRTYVGPMTESLFPGYHTKARAVMNFVVRYRPDEQPSLRPHHDSSTFTLNVALNHKGLDYEGGGCRFLRYDCVISSPRKGWALLHPGRLTHYHEGLPTTWGTRYIMVSFVDP

SEQ ID NO: 18 - DNA, 4713 bp, synthetic construct
  source 1..4713: mol_type = other DNA
atggcaacaacacttattagtaaactcactctttctagtgcttttcttggacagcaattttctagcaggggaaattctatgagaagtgctccagccggtttatttttgcgcggtcctagaatggatataagtaacttgccaccacatattagacagcaaattcttggtcttatctcaaagcctcaacagaacaatgatgaatcttcatcatctaataataagaataatcttatcaataacgaaaaggtttctaatgttcttattgatcttacttctaatttgaagattgaaaattttaaaatttttaataaagagtcacttaatcaactcgaaaaaaagggatacctcataattgataatttcttaaatgaccttaataagattaatcttatttatgatgaatcttataaccaatttaaggaaaacaagcttattgaagctggtatgaataagggtacagataaatggaaagataagagtattagaggggattatattcagtggattcatagagattccaattctagaattcaagataaggatctttcaagtacaattagaaatattaattatttgttggacaagttggatcttattaagaatgagtttgataacgttatccctaattttaattctatcaagactcaaacccaattggctgtatatttgaacggaggaagatacattaaacatagggatagtttttattcctcagaatctttgactattagcagaagaattactatgatttattatgtcaataaagactggaaaaagggagatggaggagagcttagactgtacactaataacccaaacaatactaatcaaaaagagttgaaacaaactgaagaatttattgatatagaaccaatagcagacagattgcttatttttttgtctccatttcttgaacatgaggttcttcaatgtaattttgaaccacgtattgctattactacatggatttatggatctggcgagggtaggggttcactccttacttgtgaggatgttgaagagaatcctggaccagcaccagatgaggaagatcatgttttggttcttcataaaggaaattttgatgaagctttggctgctcacaaatatttgcttgttgaattctatgctccttggtgtggtcattgcaaggcattggcccctgagtatgctaaggcagctggaaagttgaaggccgagggatctgaaattagacttgcaaaggttgacgctactgaggaatctgatttggcacaacaatatggtgttagaggttacccaactattaagttctttaagaatggtgacactgctagtcctaaggaatataccgctggtagagaggccgatgatatcgtaaattggcttaagaaaaggacaggaccagcagcttcaacattgtcagatggtgctgctgctgaagctttagtcgaatcttcagaagttgctgtgattggattttttaaagacatggaatctgatagtgccaaacagttttttttggctgcagaggtgattgatgatattccatttggaattacttcaaattcagatgtgttttcaaaatatcagcttgataaggacggagttgttttgttcaaaaagttcgatgaaggaagaaataattttgaaggtgaagtgactaaagaaaagcttcttgattttattaagcacaatcaattgccattggttattgaatttactgagcaaactgctccaaagatttttggtggtgaaattaagactcatattcttttgttcttgcctaagtctgttagtgattatgaaggtaagttgagcaactttaaaaaggctgctgaatcttttaagggaaaaattctttttatcttcattgatagcgatcacacagataatcagagaatattggaattcttcggtttgaagaaggaagaatgccctgctgttaggttgattacactggaggaggagatgactaagtacaagcctgaatctgatgagcttactgctgaaaagatcactgaattctgccacagatttcttgaggggaagattaagccacaccttatgtctcaggagttacctgatgattgggataaacaacctgttaaggttctcgtgggtaagaactttgaagaggttgctttcgatgaaaaaaaaaatgttttcgttgaattctatgcaccttggtgcggtcattgtaaacagctagcaccaatttgggataaacttggggaaacttataaggatcatgagaatattgttatagctaaaatggattcaacggctaatgaagttgaagctgttaaagtccattcatttcctactcttaagttctttcctgcttcagcagaccgtaccgttattgattacaatggtgagagaacattggatggctttaaaaaatttttggaatctggcggacaggatggagctggagatgatgatgacttggaggatttagaggaggccgaagagcctgatttggaagaagatgatgatcaaaaagcagtgaaggatgaactaggttcaggagagggtagggggagtttgttgacttgcgaggatgtagaagaaaaccctggtccatctgatagacctagaggtagagatcctgttaacccagagaagcttttggttattacagtggctacagctgagacagaaggatatcttaggtttctaaggtctgctgaattttttaattatacagttagaacattgggacttggggaggaatggagaggtggggatgttgctcgaactgtgggaggaggtcaaaaggttcgttggttgaagaaagaaatggaaaaatatgcagatagagaagatatgattattatgtttgttgatagttacgatgttattttggctggaagccctacagaattgttaaagaagtttgttcaatctggctcaaggcttttgttctccgcagagagtttctgctggccagagtggggactagctgaacagtatcctgaggtgggtactggtaagaggtttctcaattccggtggttttattggcttcgcaactactattcaccaaattgttagacaatggaagtataaagatgatgatgatgatcaacttttttatacaagactttaccttgacccaggtttgagagaaaagttgtctctgaacttggatcacaagtctagaattttccaaaatctcaatggagctttggatgaagttgttttgaaatttgatagaaatagggttaggattcgtaatgttgcctatgacacacttcctattgtagtgcatggaaatggacctactaagcttcagttgaactatttaggtaactatgtgcctaacggatggactccagaaggtggttgtggattttgtaatcaagatcgaagaactttgccaggaggacaacctccaccaagggtttttcttgctgttttcgttgagcaacctaccccattccttccaagattcttacaaagacttttgttgcttgattatccaccagatagagttactttgttccttcacaataatgaggtgtttcatgagcctcatattgctgatagttggccacaactccaagatcatttctccgcagttaagctcgttggtccagaggaagctttgtctcctggtgaagctagggatatggcaatggatctttgcagacaagatcctgaatgcgaattttacttttctttggatgctgatgctgtgcttacaaatcttcagactctaagaattttgatagaggagaacaggaaagttattgctccaatgcttagtaggcatggtaaattgtggagtaatttctggggagctctttctccggatgaatattatgctagatcggaagattacgtggagcttgttcaacgtaagagagttggtgtatggaatgttccatatatctcacaagcttacgttatcagaggagatacattgagaatggaacttcctcagagagatgtttttagcggatcagataccgatcctgatatggcattttgtaaatcattcagagataagggaattttccttcatctatctaatcagcacgaattcggaaggttgcttgctacatcaagatatgatactgagcacctgcatccagatttgtggcaaattttcgataatccagtggattggaaagaacaatacatacatgaaaattattctagagctcttgaaggtgagggaattgtcgaacaaccttgcccagacgtctattggtttccacttctttctgagcaaatgtgcgatgaactagtggcagagatggaacattacggacaatggtctggaggacggcatgaggattcaagattggctggagggtacgagaatgtgccaactgtcgatattcatatgaagcaagttggatatgaagatcagtggttgcaacttttaagaacatacgttggtcctatgactgaatcattgtttccaggataccacacaaaagcaagagcagttatgaatttcgttgttagatacagaccagatgagcaaccttctttaagaccacatcatgattcttctacatttactctcaatgttgctttgaatcacaaaggtcttgattatgagggaggaggatgcaggtttctgagatatgattgtgtaatttcatcgcctcgtaaaggatgggctttgctccatccaggaagacttactcactatcatgaaggactccctactacatggggtactagatatattatggtttcatttgttgatccttga

SEQ ID NO: 19 - protein, 2831 aa, synthetic construct
MATTLISKLTLSSAFLGQQFSSRGNSMRSAPAGLFLRGPRARAGSGQQGPGQQGPGQQGPGQQGPYGPGASAAAAAAGGYGPGSGQQGPSQQGPGQQGPGGQGPYGPGASAAAAAAGGYGPGSGQQGPGGQGPYGPGSSAAAAAAGGNGPGSGQQGAGQQGPGQQGPGASAAAAAAGGYGPGSGQQGPGQQGPGGQGPYGPGASAAAAAAGGYGPGSGQGPGQQGPGGQGPYGPGASAAAAAAGGYGPGSGQQGPGQQGPGQQGPGGQGPYGPGASAAAAAAGGYGPGYGQQGPGQQGPGGQGPYGPGASAASAASGGYGPGSGQQGPGQQGPGGQGPYGPGASAAAAAAGGYGPGSGQQGPGQQGPGQQGPGQQGPGGQGPYGPGASAAAAAAGGYGPGSGQQGPGQQGPGQQGPGQQGTYPEHEREPGQQGPGQQGPGQQGPGQQGPGQQGPGGQGAYGPGASAAAGAAGGYGPGSGQQGPGQQGPGQQGPGQQGPGQQGPGQQGPGQQGPGQQGPYGPGASAAAAAAGGYGPGSGQQGPGQQGPGQQGPGGQGPYGPGAASAAVSVGGYGPQSSSVPVASAVASRLSSPAASSRVSSAVSSLVSSGPTKHAALSNTISSVVSQVSASNPGLSGCDVLVQALLEVVSALVSILGSSSIGQINYGASAQYTQMVGQSVAQALAGSGEGRGSLLTCEDVEENPGPQLSYGYDEKSTGGISVPGPMGPSGPRGLPGPPGAPGPQGFQGPPGEPGEPGASGPMGPRGPPGPPGKNGDDGEAGKPGRPGERGPPGPQGARGLPGTAGLPGMKGHRGFSGLDGAKGDAGPAGPKGEPGSPGENGAPGQMGPRGLPGERGRPGAPGPAGARGNDGATGAAGPPGPTGPAGPPGFPGAVGAKGEAGPQGPRGSEGPQGVRGEPGPPGPAGAAGPAGNPGADGQPGAKGANGAPGIAGAPGFPGARGPSGPQGPGGPPGPKGNSGEPGAPGSKGDTGAKGEPGPVGVQGPPGPAGEEGKRGARGEPGPTGLPGPPGERGGPGSRGFPGADGVAGPKGPAGERGSPGPAGPKGSPGEAGRPGEAGLPGAKGLTGSPGSPGPDGKTGPPGPAGQDGRPGPPGPPGARGQAGVMGFPGPKGAAGEPGKAGERGVPGPPGAVGPAGKDGEAGAQGPPGPAGPAGERGEQGPAGSPGFQGLPGPAGPPGEAGKPGEQGVPGDLGAPGPSGARGERGFPGERGVQGPPGPAGPRGANGAPGNDGAKGDAGAPGAPGSQGAPGLQGMPGERGAAGLPGPKGDRGDAGPKGADGSPGKDGVRGLTGPIGPPGPAGAPGDKGESGPSGPAGPTGARGAPGDRGEPGPPGPAGFAGPPGADGQPGAKGEPGDAGAKGDAGPPGPAGPAGPPGPIGNVGAPGAKGARGSAGPPGATGFPGAAGRVGPPGPSGNAGPPGPPGPAGKEGGKGPRGETGPAGRPGEVGPPGPPGPAGEKGSPGADGPAGAPGTPGPQGIAGQRGVVGLPGQRGERGFPGLPGPSGEPGKQGPSGASGERGPPGPMGPPGLAGPPGESGREGAPGAEGSPGRDGSPGAKGDRGETGPAGPPGAPGAPGAPGPVGPAGKSGDRGETGPAGPAGPVGPVGARTYPEHEREGPAGPQGPRGDKGETGEQGDRGIKGHRGFSGLQGPPGPPGSPGEQGPSGASGPAGPRGPPGSAGAPGKDGLNGLPGPIGPPGPRGRTGDAGPVGPPGPPGPPGPPGPPSAGFDFSFLPQPPQEKAHDGGRYYRAGSGEGRGSLLTCEDVEENPGPQYDGKGVGLGPGPMGLMGPRGPPGAAGAPGPQGFQGPAGEPGEPGQTGPAGARGPAGPPGKAGEDGHPGKPGRPGERGVVGPQGARGFPGTPGLPGFKGIRGHNGLDGLKGQPGAPGVKGEPGAPGENGTPGQTGARGLPGERGRVGAPGPAGARGSDGSVGPVGPAGPIGSAGPPGFPGAPGPKGEIGAVGNAGPAGPAGPRGEVGLPGLSGPVGPPGNPGANGLTGAKGAAGLPGVAGAPGLPGPRGIPGPVGAAGATGARGLVGEPGPAGSKGESGNKGEPGSAGPQGPPGPSGEEGKRGPNGEAGSAGPPGPPGLRGSPGSRGLPGADGRAGVMGPPGSRGASGPAGVRGPNGDAGRPGEPGLMGPRGLPGSPGNIGPAGKEGPVGLPGIDGRPGPIGPAGARGEPGNIGFPGPKGPTGDPGKNGDKGHAGLAGARGAPGPDGNNGAQGPPGPQGVQGGKGEQGPPGPPGFQGLPGPSGPAGEVGKPGERGLHGEFGLPGPAGPRGERGPPGESGAAGPTGPIGSRGPSGPPGPDGNKGEPGVVGAVGTAGPSGPSGLPGERGAAGIPGGKGEKGEPGLRGEIGNPGRDGARGAPGAVGAPGPAGATGDRGEAGAAGPAGPAGPRGSPGERGEVGPAGPNGFAGPAGAAGQPGAKGERGAKGPKGENGVVGPTGPVGAAGPAGPNGPPGPAGSRGDGGPPGMTGFPGAAGRTGPPGPSGISGPPGPPGPAGKEGLRGPRGDQGPVGRTGEVGAVGPPGFAGEKGPSGEAGTAGPPGTPGPQGLLGAPGILGLPGSRGERGLPGVAGAVGEPGPLGIAGPPGARGPPGAVGSPGVNGAPGEAGRDGNPGNDGPPGRDGQPGHKGERGYPGNIGPVGAAGAPGPHGPVGPAGKHGNRGETGPSGPVGPAGAVGPRGPSGPQGIRGDKGEPGEKGPRGLPGLKGHNGLQGLPGIAGHHGDQGAPGSVGPAGPRGPAGPSGPAGKDGRTGHPGTVGPAGIRGPQGHQGPAGPPGPPGPPGPPGVSGGGYDFGYDGDFYRA

SEQ ID NO: 20 - DNA, 8448 bp, synthetic construct
  source 1..8448: mol_type = other DNA
atggctactactttgatttcaaagttaaccctttctagtgctttcctcggccaacagttttcttctaggggtaattctatgagatctgcacctgcaggattgtttcttcgtggaccaagagctagagcaggatcgggtcaacaaggaccaggacaacagggaccaggacaacagggtccaggtcaacaaggaccatatggtcctggagcatcagcagctgctgctgcagctggtggatacggtccaggaagcggtcaacaaggtccatcccaacaaggtcctggtcaacaaggaccaggagggcaaggtccttacggacctggtgctagtgcagctgctgcagctgctggaggttacggaccaggttctggtcaacaaggaccaggaggacaaggtccatacggaccaggatcttctgctgcagctgctgctgcaggaggaaatggtcctggatctggacaacaaggagcaggtcaacaaggtcctggccaacaaggtccaggtgcttctgctgctgctgctgcagcaggtggttatggtcccggatcaggacaacaaggtcctggacaacaaggtcctggaggacaaggaccttatggtcctggtgctagtgctgctgctgctgctgctggaggatatggtccaggaagcggacaaggaccaggacagcaagggcctggaggtcagggtccatatggtcctggagcttctgcagctgctgctgctgctggtggatatggaccaggttctggacaacagggtcctggtcaacaaggaccaggacagcagggaccaggaggtcaaggtccatatggacctggagcatcagcagctgcagcagctgcaggtggctatggtcctggatatggtcaacagggacctggacagcagggtcctggaggtcaaggtccttatggtcctggagcttcagctgcttctgcagcttccggtggatatggacctggatctggtcagcaaggccctggtcaacaaggtccaggaggtcaaggaccttatgggcctggagcttctgctgctgcagctgcagctggaggatacggacctggatctggtcagcaaggaccaggtcaacagggtccaggtcaacaaggaccaggtcaacaaggtccaggagggcagggaccatatggacctggagcttcagcagcagctgctgctgctggtggatacggtccaggttcaggacaacagggccctggacaacaaggacctggccaacaaggacctggtcaacaaggtcctggtcaacaaggacctggtcaacaaggaccaggacaacaaggaccaggtcaacagggaccaggtcaacaaggtcctggaggtcagggtgcttatggtccaggtgcttccgctgctgctggtgctgcaggtggttacggacctggatctggacagcaaggaccaggtcaacaaggacctggacaacaaggtccaggacaacaaggacctggacaacaaggtccaggtcaacaaggtcctggtcagcagggtccaggacaacaaggtccttatggaccaggggctagcgctgctgcagcagcagcaggtggatatggaccaggtagtggtcaacaaggtcctggacagcaaggtcctggtcaacaaggtcctggaggtcaaggaccctacggtccaggtgctgcttcagcagctgtgtctgttggtggatatggaccacagtcttcttcagtcccagttgcatctgcagttgcatctagactttcatctccagctgcttcatctagagtttcttctgctgtttcttctcttgtgtcatctggtccaactaaacatgctgcactttctaacacaattagttcagttgtttctcaagtttctgcatctaacccaggactttctggttgcgatgttcttgtgcaagctcttctggaagttgttagtgctttggtttccattttgggttctagctctattggacagatcaattatggtgcttcagcacaatacactcaaatggttggacaaagcgttgctcaggctcttgctggaagcggagaaggaagaggtagtctgcttacatgtgaagatgttgaagaaaatcctggtccacaactttcatatggttatgatgagaaatcaacaggtggtatttctgtgccaggacctatgggtccttcaggccctagaggattgccaggtccacctggtgctcctggtcctcaaggattccaaggaccaccaggtgagccaggtgaacctggagctagtggaccaatgggtcctagaggtccacctggtcctcctggtaaaaatggtgatgatggagaggcaggaaagcctggaagacctggagaaagaggaccacctggacctcaaggagctcggggacttccaggtacagctggattgccaggtatgaagggacacagaggattcagtggcttggatggagctaagggagatgctggtccagctggacctaaaggagagccaggttctccaggagaaaacggagctccaggacaaatgggacctagaggtcttcctggtgaaaggggtaggccaggagcccctggacctgctggtgctagaggtaacgatggagctactggtgctgctggaccaccaggacctactggtcctgcaggtccaccaggttttccaggtgcagttggagcaaagggtgaggctggtccacaaggacctagaggttcagaaggaccacaaggtgttagaggtgaaccaggtccaccgggaccagcaggagccgctggccccgctggtaatcctggtgctgatggtcaaccaggtgctaagggagctaacggtgctccagggattgctggtgctccaggattccctggagctagaggaccttcaggtccacaaggtcctggtggaccacctggaccaaaaggaaatagcggagagccaggtgcacctggctcaaagggagatactggagcaaagggagagcctggacctgttggtgttcaaggtcctcctggacctgctggtgaggagggaaagagaggtgcaagaggtgagcctggtcctacaggactccctggtcctcctggtgaaaggggaggacctggatctaggggttttccaggtgctgatggagttgctggacctaaaggaccagctggagaaaggggatctccaggtccagctgggccaaagggttctcctggagaggcaggaagaccaggtgaagctggattgccaggtgccaagggacttacaggatctcctgggtcaccaggaccagatggaaagactggtcctcctggaccagctggacaagatggaagacctggaccacctggaccacctggagcaaggggtcaagctggtgttatgggttttccaggtccaaaaggtgcagcaggcgagccaggaaaggctggtgaaaggggtgttccaggtccacctggagcagttggtccagctggaaaggatggagaggctggcgctcaaggtcctcctggtcctgctgggccagcaggtgaaagaggagaacaaggacctgctgggtctcctggttttcaaggacttcctggaccagctggtcctccaggtgaagcaggcaagccaggagagcaaggtgttcctggagatcttggtgccccaggtccttctggtgcaagaggagagcgtggattccctggagaaagaggtgtgcaaggtcctccaggtccagctggtccacgtggagctaacggagctcctggtaacgatggagctaaaggagatgctggtgccccaggcgcacctggttcacaaggtgctcctggattgcaaggtatgcctggcgaaagaggtgctgctggacttcctggacctaagggtgacagaggtgatgctggaccaaaaggagctgatggatcacctggtaaagatggagtgagaggtttaaccggtccaattggaccaccaggtcccgctggagctccaggagataaaggagaaagtggaccatcaggtcctgccggtcccactggtgctagaggtgcacctggtgatagaggtgaacctggtccaccagggcctgctggatttgctggtccaccaggagcagatggacaaccaggagcaaaaggtgagcctggagatgctggagctaaaggagatgcaggtcctcctggaccagctggacctgctggaccacctggaccaattggaaatgttggtgctccaggagctaaaggggcaagaggatctgctggtcctcctggagcaactgggttccctggagcagcaggaagagttggtcctcctggaccttctggaaacgctggacctcctggtccaccaggacctgctggaaaggaaggaggaaagggtccaagaggcgaaactggaccagcaggtagaccaggagaggttggaccacctggaccacctggtcccgctggagagaaaggatctcctggagctgatggaccagcaggtgctccaggcactccaggcccacaaggaattgctggtcaaaggggagttgttggattgcctgggcaaagaggagagaggggatttcctggtcttcctggtccatcaggtgaacctggaaaacaaggtccatctggagctagtggtgagaggggccctccaggaccaatgggcccacctggacttgctggacctcctggagagtccggtagagaaggggctccaggtgctgaaggatcaccaggaagggatggatctcctggagccaagggggatagaggagaaacaggtccagcagggcctcctggtgcaccaggtgcacctggtgctcctggtccagttggacctgcaggtaaatctggtgatcgtggagaaactggtccagctggacctgctggacctgttggaccagtgggtgctcgtggacctgctggtccacagggaccaagaggagataaaggtgagactggtgagcaaggtgatagaggaattaaaggacataggggtttttctggcttacagggtcctccaggtccaccaggatctccaggagaacaaggtccatcaggagctagtggaccagcagggccaaggggacctcctggttctgctggtgcaccaggtaaagatgggcttaacggattgcctggacctataggtcctccaggtccaagaggaagaactggtgatgctggtcctgttggaccaccaggtccacctggaccaccagggccacctggacctccatctgcaggatttgatttttctttccttccacaaccaccacaagaaaaggctcacgatggtggaaggtattatagggcaggctctggtgaagggcgtggaagtcttcttacatgtgaggatgttgaagaaaatccaggaccacaatatgatggaaagggtgttggattgggtccaggtccaatgggattgatgggccctagaggtcctcctggagctgctggagctcctggaccacaaggattccagggcccagctggtgaacctggagaaccgggacaaacaggaccagctggtgctagaggtccagctggtcctccaggaaaagctggagaagatggccatcctggtaaaccaggtaggccaggagaaagaggtgttgtgggtccacagggagctaggggatttcctggtactcctgggttgcctggattcaagggaattaggggtcataatggtcttgatggtcttaaaggacaaccaggagctcctggtgttaaaggagaacctggagcacctggtgaaaatggtactccaggtcaaacaggtgcaagaggattgccaggagaaaggggtagagtgggagcaccaggtcctgctggagctagaggttcagatggaagtgtgggacctgtgggacctgcaggaccaattggatcagctggtccacctggatttccaggtgccccaggtccaaagggagaaattggagctgttggaaatgcgggcccagcaggcccagctggacctagaggtgaggttggtctaccaggtctgtcaggaccagtgggccctccaggaaatcctggtgcaaatgggcttacaggagctaagggagcagctggattgcctggtgttgctggggcaccaggtcttcctggtccaagaggtattccaggaccagtaggtgctgcaggagcaactggagctagaggtttggttggtgaaccaggaccagcaggctccaagggtgaatctggtaataagggagaacctggttctgctggaccacaaggaccaccaggaccatcaggagaagaaggtaagaggggtcctaacggagaggccggttctgcaggtccacctggaccacctggacttagaggatctccagggtctagaggtttacctggtgctgatggtagagctggagtgatgggtcctccaggttcaagaggagcatctggcccagcaggagttaggggaccaaatggtgatgctgggagaccaggtgaaccaggtcttatgggtcctagaggattgccaggttcaccaggaaatattggtccagctggaaaagaaggaccagttggacttcctggaattgatggtagaccaggtcctattggtcctgctggtgctagaggtgagccaggtaatatcggttttccaggaccaaagggaccaactggtgatccaggcaaaaatggtgataagggacatgctggactcgcaggagctagaggcgctccaggacctgatggaaataatggtgcccagggacctccaggaccacaaggtgttcaaggaggaaagggtgagcaaggacctccaggacctccaggttttcagggacttccaggaccatctggaccagcaggtgaggttggtaagccaggagaaaggggtttacatggtgaattcggtctgccaggaccagctggaccaaggggtgaaaggggtccaccaggagagtcaggtgctgctggaccaacaggaccaattggttcaagaggtccatctggacctccaggtcctgatggaaacaaaggtgaaccaggagttgtaggtgctgttggaactgctggtccttcaggcccaagcggacttccaggtgaaaggggtgctgctggtattcctggaggtaagggtgaaaaaggggagcctggtcttagaggtgagattggtaatccaggaagagatggggctagaggtgcaccaggagccgttggtgctcctggtcctgctggagctacaggagatagaggagaggcaggagctgctggtcctgctggaccagctggcccaagaggtagcccaggagaaagaggtgaagttggtccagctggtcctaatggatttgctggacctgctggtgctgctggtcagcctggagctaaaggggaaagaggagccaaaggacctaaaggagaaaatggagttgttgggcctacaggaccagtaggagcagcaggacctgctggtccaaatggaccaccaggaccagcaggatccagaggagatggtggtccaccaggaatgacaggttttcctggtgctgctggaagaacaggaccaccaggtccttcaggtatttctggtcctccaggtcctccaggaccagctggaaaggagggtttgagaggacctagaggtgatcaaggacctgtgggaagaacaggagaagttggagcagttggaccaccaggtttcgctggagaaaagggaccatctggcgaagctggaactgctggaccaccaggtacccctggacctcagggacttcttggagctcctggaattttgggacttcccggatctagaggagagaggggattgccaggcgttgctggagctgtgggtgagccaggtcctctcggaattgctggaccacctggtgcaaggggtccaccaggtgccgttgggtccccaggtgttaatggtgctccaggtgaggctggtagggatggaaatccaggtaatgatggaccacctggtagggatggacagcctggccataagggtgagcgtggatatccaggtaatattggaccagttggtgcagcaggggcaccaggaccacacggacctgttggtccagctggtaagcacggcaataggggagagactggtccttcaggacctgtgggtccggctggagcagttggacctagaggtccatcaggaccacaaggaattagaggtgataagggagaacccggggagaaaggaccaagaggattacctggattaaagggtcacaatggattacaaggattgcctggaattgctggacatcacggagatcaaggagcaccaggatcagttggaccggctggaccaagaggacctgcaggaccttctggacctgctggtaaagatggaagaactggacatcctggtacagttggacctgctggaattagaggtccacaaggtcatcaagggcctgccggtcctccaggaccaccaggaccaccagggcctccaggagtttctggcggtggatatgattttggttatgatggagatttttaccgtgcttga